European Patent Specification EP 3 813 870 B1, published November 15, 2023. Title: METHODS OF TREATING CANCER. Applicant: ORION Biotechnology Switzerland Sàrl. The sequence listing filed with the application follows.

SEQUENCE LISTING (72 sequences)

SEQ ID NO: 1 - protein, 59 aa, Homo sapiens
CCFAYIARPLPRAHIKEYFYTSGKCSNPAVVFVTRKNRQVCANPEKKWVREYINSLEMS

SEQ ID NO: 2 - protein, 10 aa, Artificial Sequence
  synthetic
QGPPLMALQS

SEQ ID NO: 3 - protein, 10 aa, Artificial Sequence
  synthetic
QGPPLMWMQV

SEQ ID NO: 4 - protein, 10 aa, Artificial Sequence
  synthetic
QGPPLMWLQV

SEQ ID NO: 5 - protein, 10 aa, Artificial Sequence
  synthetic
QGPPLMWTQS

SEQ ID NO: 6 - protein, 10 aa, Artificial Sequence
  synthetic
QGPPLMWLQT

SEQ ID NO: 7 - protein, 10 aa, Artificial Sequence
  synthetic
QGPPLMWTQV

SEQ ID NO: 8 - protein, 10 aa, Artificial Sequence
  synthetic
QGPPLMWMQS

SEQ ID NO: 9 - protein, 10 aa, Artificial Sequence
  synthetic
QGPPLMATQS

SEQ ID NO: 10 - protein, 10 aa, Artificial Sequence
  synthetic
QGPPLMWLQS

SEQ ID NO: 11 - protein, 10 aa, Artificial Sequence
  synthetic
QGPPLMALQV

SEQ ID NO: 12 - protein, 10 aa, Artificial Sequence
  synthetic
QGPPLMWLGG

SEQ ID NO: 13 - protein, 10 aa, Artificial Sequence
  synthetic
QGPPLMWRGS

SEQ ID NO: 14 - protein, 10 aa, Artificial Sequence
  synthetic
QGPLLMWLQV

SEQ ID NO: 15 - protein, 10 aa, Artificial Sequence
  synthetic
QGPPLMQTTP

SEQ ID NO: 16 - protein, 10 aa, Artificial Sequence
  synthetic
QGPPGDTVLW

SEQ ID NO: 17 - protein, 10 aa, Artificial Sequence
  synthetic
QGPPGDIVLA

SEQ ID NO: 18 - protein, 10 aa, Artificial Sequence
  synthetic
QGPPGSYDYS

SEQ ID NO: 19 - protein, 10 aa, Artificial Sequence
  synthetic
QGPPGDGGSV

SEQ ID NO: 20 - protein, 10 aa, Artificial Sequence
  synthetic
QGPLSGQSTP

SEQ ID NO: 21 - protein, 10 aa, Artificial Sequence
  synthetic
QGPPGDWLQV

SEQ ID NO: 22 - protein, 10 aa, Artificial Sequence
  synthetic
QGPPLMSFQS

SEQ ID NO: 23 - protein, 10 aa, Artificial Sequence
  synthetic
QGPPLMSTQS

SEQ ID NO: 24 - protein, 10 aa, Artificial Sequence
  synthetic
QGPPLMSLQV

SEQ ID NO: 25 - protein, 10 aa, Artificial Sequence
  synthetic
QGPPLMGLQV

SEQ ID NO: 26 - protein, 10 aa, Artificial Sequence
  synthetic
QGPLSGWLQV

SEQ ID NO: 27 - protein, 10 aa, Artificial Sequence
  synthetic
QGPPLMSVLA

SEQ ID NO: 28 - protein, 10 aa, Artificial Sequence
  synthetic
QGPPGSWSSV

SEQ ID NO: 29 - protein, 10 aa, Artificial Sequence
  synthetic
QGPPLGSMGP

SEQ ID NO: 30 - protein, 10 aa, Artificial Sequence
  synthetic
QGPPLSWLQV

SEQ ID NO: 31 - protein, 10 aa, Artificial Sequence
  synthetic
QGPPLSWLQS

SEQ ID NO: 32 - protein, 10 aa, Artificial Sequence
  synthetic
QGPPGQWSQV

SEQ ID NO: 33 - protein, 10 aa, Artificial Sequence
  synthetic
QGPPMMAGLS

SEQ ID NO: 34 - protein, 10 aa, Artificial Sequence
  synthetic
QGPPLSWQQS

SEQ ID NO: 35 - protein, 10 aa, Artificial Sequence
  synthetic
QGPPGMWSQS

SEQ ID NO: 36 - protein, 10 aa, Artificial Sequence
  synthetic
QGPPLQWRQS

SEQ ID NO: 37 - protein, 10 aa, Artificial Sequence
  synthetic
QGPPLMGTQS

SEQ ID NO: 38 - protein, 10 aa, Artificial Sequence
  synthetic
QGPPLMQLQV

SEQ ID NO: 39 - protein, 10 aa, Artificial Sequence
  synthetic
QGPPLSWSQV

SEQ ID NO: 40 - protein, 10 aa, Artificial Sequence
  synthetic
QGPPMSWSQS

SEQ ID NO: 41 - protein, 10 aa, Artificial Sequence
  synthetic
QGPPLMNLQV

SEQ ID NO: 42 - protein, 10 aa, Artificial Sequence
  synthetic
QGPPMSAYQV

SEQ ID NO: 43 - protein, 10 aa, Artificial Sequence
  synthetic
QGPPMQGGLS

SEQ ID NO: 44 - protein, 10 aa, Artificial Sequence
  synthetic
QGPPLMSLAV

SEQ ID NO: 45 - protein, 10 aa, Artificial Sequence
  synthetic
QGPPLMSLTV

SEQ ID NO: 46 - protein, 10 aa, Artificial Sequence
  synthetic
QGPLSGWAQV

SEQ ID NO: 47 - protein, 10 aa, Artificial Sequence
  synthetic
QGPLSQSSQV

SEQ ID NO: 48 - protein, 10 aa, Artificial Sequence
  synthetic
QGPLSSQSQV

SEQ ID NO: 49 - protein, 10 aa, Artificial Sequence
  synthetic
QGPLGQQGQV

SEQ ID NO: 50 - protein, 10 aa, Artificial Sequence
  synthetic
QGPPLQWFQV

SEQ ID NO: 51 - protein, 10 aa, Artificial Sequence
  synthetic
QGPPLQWTQV

SEQ ID NO: 52 - protein, 10 aa, Artificial Sequence
  synthetic
QGPPLMALSV

SEQ ID NO: 53 - protein, 10 aa, Artificial Sequence
  synthetic
QGPPLMWSQV

SEQ ID NO: 54 - protein, 10 aa, Artificial Sequence
  synthetic
QGPPGQWGQV

SEQ ID NO: 55 - protein, 10 aa, Artificial Sequence
  synthetic
QGPPGSWSQV

SEQ ID NO: 56 - protein, 10 aa, Artificial Sequence
  synthetic
QGPPLMSSQS

SEQ ID NO: 57 - protein, 10 aa, Artificial Sequence
  synthetic
QGPPLMGLSV

SEQ ID NO: 58 - protein, 10 aa, Artificial Sequence
  synthetic
QGPPLMTLQV

SEQ ID NO: 59 - protein, 10 aa, Artificial Sequence
  synthetic
QGPPGQWYQS

SEQ ID NO: 60 - protein, 10 aa, Artificial Sequence
  synthetic
QGPPLQWMQA

SEQ ID NO: 61 - protein, 10 aa, Artificial Sequence
  synthetic
QGPPLQWMQV

SEQ ID NO: 62 - protein, 10 aa, Artificial Sequence
  synthetic
QGPPLMSTQV

SEQ ID NO: 63 - protein, 10 aa, Artificial Sequence
  synthetic
QGPPLMSLSV

SEQ ID NO: 64 - protein, 10 aa, Artificial Sequence
  synthetic
QGPPLMSLQS

SEQ ID NO: 65 - protein, 10 aa, Artificial Sequence
  synthetic
QGPPLMSLQA

SEQ ID NO: 66 - protein, 10 aa, Artificial Sequence
  synthetic
QGPPLMSVQS

SEQ ID NO: 67 - protein, 10 aa, Artificial Sequence
  synthetic
QGPPLMSAQS

SEQ ID NO: 68 - protein, 10 aa, Artificial Sequence
  synthetic
QGPPLMSGQS

SEQ ID NO: 69 - protein, 10 aa, Artificial Sequence
  synthetic
QGPPLMSGQV

SEQ ID NO: 70 - protein, 69 aa, Artificial Sequence
  synthetic
QGPPLMATQSCCFAYIARPLPRAHIKEYFYTSGKCSNPAVVFVTRKNRQVCANPEKKWVREYINSLEMS

SEQ ID NO: 71 - protein, 69 aa, Artificial Sequence [sequence omitted]

SEQ ID NO: 72 - protein, 69 aa, Artificial Sequence
  synthetic
QGPPLMSLQVCCFAYIARPLPRAHIKEYFYTSGKCSNPAVVFVTRKNRQVCANPEKKWVREYINSLEMS